European Patent Application EP 4 218 804 A2, published August 2, 2023. Title: USE OF MYOSTATIN INHIBITORS AND COMBINATION THERAPIES. Applicant: SCHOLAR ROCK, INC. Application EP. The sequence listing filed with the application follows.

SEQUENCE LISTING (116 sequences)

SEQ ID NO: 1 - protein, 6 aa, synthetic construct
  source 1..6: note = Synthetic
SSYGMH

SEQ ID NO: 2 - protein, 10 aa, synthetic construct
  source 1..10: note = Synthetic
GFTFSSYGMH

SEQ ID NO: 3 - protein, 10 aa, synthetic construct
  source 1..10: note = Synthetic
GFAFSSYGMH

SEQ ID NO: 4 - protein, 17 aa, synthetic construct
  source 1..17: note = Synthetic
VISYDGSNKYYADSVKG

SEQ ID NO: 5 - protein, 7 aa, synthetic construct
  source 1..7: note = Synthetic
ISYDGSN

SEQ ID NO: 6 - protein, 17 aa, synthetic construct
  source 1..17: note = Synthetic
VISYDGSIKYYADSVKG

SEQ ID NO: 7 - protein, 7 aa, synthetic construct
  source 1..7: note = Synthetic
ISYDGSI

SEQ ID NO: 8 - protein, 17 aa, synthetic construct
  source 1..17: note = Synthetic
VISYDGNNKYYADSVKG

SEQ ID NO: 9 - protein, 7 aa, synthetic construct
  source 1..7: note = Synthetic
ISYDGNN

SEQ ID NO: 10 - protein, 17 aa, synthetic construct
  source 1..17: note = Synthetic
DLLVRFLEWSHYYGMDV

SEQ ID NO: 11 - protein, 17 aa, synthetic construct
  source 1..17: note = Synthetic
DLLVRFLEWSHKYGMDV

SEQ ID NO: 12 - protein, 13 aa, synthetic construct
  source 1..13: note = Synthetic
SGSSSNIGSNTVH

SEQ ID NO: 13 - protein, 8 aa, synthetic construct
  source 1..8: note = Synthetic
SSNIGSNT

SEQ ID NO: 14 - protein, 13 aa, synthetic construct
  source 1..13: note = Synthetic
SGSTSNIGSNTVH

SEQ ID NO: 15 - protein, 8 aa, synthetic construct
  source 1..8: note = Synthetic
TSNIGSNT

SEQ ID NO: 16 - protein, 13 aa, synthetic construct
  source 1..13: note = Synthetic
SGSSSNIGGNTVH

SEQ ID NO: 17 - protein, 8 aa, synthetic construct
  source 1..8: note = Synthetic
SSNIGGNT

SEQ ID NO: 18 - protein, 7 aa, synthetic construct
  source 1..7: note = Synthetic
SDNQRPS

SEQ ID NO: 19 - skipped

SEQ ID NO: 20 - protein, 7 aa, synthetic construct
  source 1..7: note = Synthetic
SDDQRPS

SEQ ID NO: 21 - skipped

SEQ ID NO: 22 - protein, 10 aa, synthetic construct
  source 1..10: note = Synthetic
AAWDDSLNGV

SEQ ID NO: 23 - protein, 10 aa, synthetic construct
  source 1..10: note = Synthetic
AAWDESLNGV

SEQ ID NO: 24 - protein, 126 aa, synthetic construct
  source 1..126: note = Synthetic
QIQLVQSGGGVVQPGRSLRLSCAASGFTFSSYGMHWVRQAPGKGLEWVAVISYDGSNKYYADSVKGRFTISRDNSKNTLYLQMNSLRAEDTAVYYCARDLLVRFLEWSHYYGMDVWGQGTTVTVSS

SEQ ID NO: 25 - protein, 126 aa, synthetic construct
  source 1..126: note = Synthetic
QVQLVESGGGVVQPGRSLRLSCAASGFTFSSYGMHWVRQAPGKGLEWVAVISYDGSNKYYADSVKGRFTISRDNSKNTLYLQMNSLRAEDTAVYYCARDLLVRFLEWSHYYGMDVWGQGTTVTVSS

SEQ ID NO: 26 - protein, 126 aa, synthetic construct
  source 1..126: note = Synthetic
QIQLVQSGGGVVQPGRSLRLSCAASGFAFSSYGMHWVRQAPGKGLEWVAVISYDGSIKYYADSVKGRFTISRDNSKNTLYLQMNSLRAEDTAVYYCARDLLVRFLEWSHKYGMDVWGQGTTVTVSS

SEQ ID NO: 27 - protein, 126 aa, synthetic construct
  source 1..126: note = Synthetic
QVQLVESGGGVVQPGRSLRLSCAASGFAFSSYGMHWVRQAPGKGLEWVAVISYDGSIKYYADSVKGRFTISRDNSKNTLYLQMNSLRAEDTAVYYCARDLLVRFLEWSHKYGMDVWGQGTTVTVSS

SEQ ID NO: 28 - protein, 126 aa, synthetic construct
  source 1..126: note = Synthetic
QIQLVQSGGGVVQPGRSLRLSCAASGFAFSSYGMHWVRQAPGKGLEWVAVISYDGNNKYYADSVKGRFTISRDNSKNTLYLQMNSLRAEDTAVYYCARDLLVRFLEWSHKYGMDVWGQGTTVTVSS

SEQ ID NO: 29 - protein, 126 aa, synthetic construct
  source 1..126: note = Synthetic
QVQLVESGGGVVQPGRSLRLSCAASGFAFSSYGMHWVRQAPGKGLEWVAVISYDGNNKYYADSVKGRFTISRDNSKNTLYLQMNSLRAEDTAVYYCARDLLVRFLEWSHKYGMDVWGQGTTVTVSS

SEQ ID NO: 30 - protein, 109 aa, synthetic construct
  source 1..109: note = Synthetic
QPVLTQPPSASGTPGQRVTISCSGSSSNIGSNTVHWYQQLPGTAPKLLIYSDNQRPSGVPDRFSGSKSGTSASLVISGLQSDDEADYYCAAWDDSLNGVFGGGTKLTVL

SEQ ID NO: 31 - protein, 109 aa, synthetic construct
  source 1..109: note = Synthetic
QSVLTQPPSASGTPGQRVTISCSGSSSNIGSNTVHWYQQLPGTAPKLLIYSDNQRPSGVPDRFSGSKSGTSASLAISGLQSEDEADYYCAAWDDSLNGVFGGGTKLTVL

SEQ ID NO: 32 - protein, 109 aa, synthetic construct
  source 1..109: note = Synthetic
QPVLTQPPSASGTPGQRVTISCSGSTSNIGSNTVHWYQQLPGTAPKLLIYSDDQRPSGVPDRFSGSKSGTSASLVISGLQSDDEADYYCAAWDESLNGVFGGGTKLTVL

SEQ ID NO: 33 - protein, 109 aa, synthetic construct
  source 1..109: note = Synthetic
QSVLTQPPSASGTPGQRVTISCSGSTSNIGSNTVHWYQQLPGTAPKLLIYSDDQRPSGVPDRFSGSKSGTSASLAISGLQSEDEADYYCAAWDESLNGVFGGGTKLTVL

SEQ ID NO: 34 - protein, 109 aa, synthetic construct
  source 1..109: note = Synthetic
QPVLTQPPSASGTPGQRVTISCSGSSSNIGGNTVHWYQQLPGTAPKLLIYSDDQRPSGVPDRFSGSKSGTSASLVISGLQSDDEADYYCAAWDESLNGVFGGGTKLTVL

SEQ ID NO: 35 - protein, 109 aa, synthetic construct
  source 1..109: note = Synthetic
QSVLTQPPSASGTPGQRVTISCSGSSSNIGGNTVHWYQQLPGTAPKLLIYSDDQRPSGVPDRFSGSKSGTSASLAISGLQSEDEADYYCAAWDESLNGVFGGGTKLTVL

SEQ ID NO: 36-37 - skipped (2 entries)

SEQ ID NO: 38 - DNA, 378 bp, synthetic construct
  source 1..378: mol_type = other DNA; note = Synthetic
cagatccagctggtgcagtctgggggaggcgtggtccagcctgggaggtccctgagactctcctgtgcagcgtctggattcaccttcagtagctatggcatgcactgggtccgccaggctccaggcaaggggctggagtgggtggcagttatatcatatgatggaagtaataaatactatgcagactccgtgaagggccgattcaccatctccagagacaattccaagaacacgctgtatctgcaaatgaacagcctgagagccgaggacacggctgtgtattactgtgcgagagatctcctggtgcgatttttggagtggtcgcactactacggtatggacgtctggggccaagggaccacggtcaccgtctcctca

SEQ ID NO: 39 - DNA, 378 bp, synthetic construct
  source 1..378: mol_type = other DNA; note = Synthetic
caggtgcagctggtggagtctgggggaggcgtggtccagcctgggaggtccctgagactctcctgtgcagcgtctggattcaccttcagtagctatggcatgcactgggtccgccaggctccaggcaaggggctggagtgggtggcagttatatcatatgatggaagtaataaatactatgcagactccgtgaagggccgattcaccatctccagagacaattccaagaacacgctgtatctgcaaatgaacagcctgagagccgaggacacggctgtgtattactgtgcgagagatctcctggtgcgatttttggagtggtcgcactactacggtatggacgtctggggccaagggaccacggtcaccgtctcctca

SEQ ID NO: 40 - DNA, 378 bp, synthetic construct
  source 1..378: mol_type = other DNA; note = Synthetic
cagatccagctggtgcagtctgggggaggcgtggtccagcctgggaggtccctgagactctcctgtgcagcgtctggattcgccttcagtagctatggcatgcactgggtccgccaggctccaggcaaggggctggagtgggtggcagttatatcatatgatggaagtatcaaatactatgcagactccgtgaagggccgattcaccatctccagagacaattccaagaacacgctgtatctgcaaatgaacagcctgagagccgaggacacggctgtgtattactgtgcgagagatctcctggtgcgatttttggagtggtcgcacaagtacggtatggacgtctggggccaagggaccacggtcaccgtctcctca

SEQ ID NO: 41 - DNA, 378 bp, synthetic construct
  source 1..378: mol_type = other DNA; note = Synthetic
caggtgcagctggtggagtctgggggaggcgtggtccagcctgggaggtccctgagactctcctgtgcagcgtctggattcgccttcagtagctatggcatgcactgggtccgccaggctccaggcaaggggctggagtgggtggcagttatatcatatgatggaagtatcaaatactatgcagactccgtgaagggccgattcaccatctccagagacaattccaagaacacgctgtatctgcaaatgaacagcctgagagccgaggacacggctgtgtattactgtgcgagagatctcctggtgcgatttttggagtggtcgcacaagtacggtatggacgtctggggccaagggaccacggtcaccgtctcctca

SEQ ID NO: 42 - DNA, 378 bp, synthetic construct
  source 1..378: mol_type = other DNA; note = Synthetic
cagatccagctggtgcagtctgggggaggcgtggtccagcctgggaggtccctgagactctcctgtgcagcgtctggattcgccttcagtagctatggcatgcactgggtccgccaggctccaggcaaggggctggagtgggtggcagttatatcatatgatggaaataataaatactatgcagactccgtgaagggccgattcaccatctccagagacaattccaagaacacgctgtatctgcaaatgaacagcctgagagccgaggacacggctgtgtattactgtgcgagagatctcctggtgcgatttttggagtggtcgcacaagtacggtatggacgtctggggccaagggaccacggtcaccgtctcctca

SEQ ID NO: 43 - DNA, 378 bp, synthetic construct
  source 1..378: mol_type = other DNA; note = Synthetic
caggtgcagctggtggagtctgggggaggcgtggtccagcctgggaggtccctgagactctcctgtgcagcgtctggattcgccttcagtagctatggcatgcactgggtccgccaggctccaggcaaggggctggagtgggtggcagttatatcatatgatggaaataataaatactatgcagactccgtgaagggccgattcaccatctccagagacaattccaagaacacgctgtatctgcaaatgaacagcctgagagccgaggacacggctgtgtattactgtgcgagagatctcctggtgcgatttttggagtggtcgcacaagtacggtatggacgtctggggccaagggaccacggtcaccgtctcctca

SEQ ID NO: 44 - DNA, 327 bp, synthetic construct
  source 1..327: mol_type = other DNA; note = Synthetic
cagcctgtgctgactcagccaccctcagcgtctgggacccccgggcagagggtcaccatctcttgttctggaagcagctccaacatcggaagtaatactgtccactggtaccagcaactcccaggaacggcccccaaactcctcatctatagtgataatcagcgcccctcaggggtccctgaccgattctctggctccaagtctggcacctcagcctccctggtcatcagtgggctccagtctgacgatgaggctgattattactgtgcagcatgggatgacagcctgaatggggtgttcggcggagggaccaagctgaccgtccta

SEQ ID NO: 45 - DNA, 327 bp, synthetic construct
  source 1..327: mol_type = other DNA; note = Synthetic
cagtctgtgctgactcagccaccctcagcgtctgggacccccgggcagagggtcaccatctcttgttctggaagcagctccaacatcggaagtaatactgtccactggtaccagcaactcccaggaacggcccccaaactcctcatctatagtgataatcagcgcccctcaggggtccctgaccgattctctggctccaagtctggcacctcagcctccctggccatcagtgggctccagtctgaggatgaggctgattattactgtgcagcatgggatgacagcctgaatggggtgttcggcggagggaccaagctgaccgtccta

SEQ ID NO: 46 - DNA, 327 bp, synthetic construct
  source 1..327: mol_type = other DNA; note = Synthetic
cagcctgtgctgactcagccaccctcagcgtctgggacccccgggcagagggtcaccatctcttgttctggaagcacctccaacatcggaagtaatactgtccactggtaccagcaactcccaggaacggcccccaaactcctcatctatagtgatgatcagcgcccctcaggggtccctgaccgattctctggctccaagtctggcacctcagcctccctggtcatcagtgggctccagtctgacgatgaggctgattattactgtgcagcatgggatgagagcctgaatggggtgttcggcggagggaccaagctgaccgtccta

SEQ ID NO: 47 - DNA, 327 bp, synthetic construct
  source 1..327: mol_type = other DNA; note = Synthetic
cagtctgtgctgactcagccaccctcagcgtctgggacccccgggcagagggtcaccatctcttgttctggaagcacctccaacatcggaagtaatactgtccactggtaccagcaactcccaggaacggcccccaaactcctcatctatagtgatgatcagcgcccctcaggggtccctgaccgattctctggctccaagtctggcacctcagcctccctggccatcagtgggctccagtctgaggatgaggctgattattactgtgcagcatgggatgagagcctgaatggggtgttcggcggagggaccaagctgaccgtccta

SEQ ID NO: 48 - DNA, 327 bp, synthetic construct
  source 1..327: mol_type = other DNA; note = Synthetic
cagcctgtgctgactcagccaccctcagcgtctgggacccccgggcagagggtcaccatctcttgttctggaagcagctccaacatcggaggaaatactgtccactggtaccagcaactcccaggaacggcccccaaactcctcatctatagtgatgatcagcgcccctcaggggtccctgaccgattctctggctccaagtctggcacctcagcctccctggtcatcagtgggctccagtctgacgatgaggctgattattactgtgcagcatgggatgagagcctgaatggggtgttcggcggagggaccaagctgaccgtccta

SEQ ID NO: 49 - DNA, 327 bp, synthetic construct
  source 1..327: mol_type = other DNA; note = Synthetic
cagtctgtgctgactcagccaccctcagcgtctgggacccccgggcagagggtcaccatctcttgttctggaagcagctccaacatcggaggaaatactgtccactggtaccagcaactcccaggaacggcccccaaactcctcatctatagtgatgatcagcgcccctcaggggtccctgaccgattctctggctccaagtctggcacctcagcctccctggccatcagtgggctccagtctgaggatgaggctgattattactgtgcagcatgggatgagagcctgaatggggtgttcggcggagggaccaagctgaccgtccta

SEQ ID NO: 50 - protein, 452 aa, synthetic construct
  source 1..452: note = Synthetic
QVQLVESGGGVVQPGRSLRLSCAASGFTFSSYGMHWVRQAPGKGLEWVAVISYDGSNKYYADSVKGRFTISRDNSKNTLYLQMNSLRAEDTAVYYCARDLLVRFLEWSHYYGMDVWGQGTTVTVSSASTKGPSVFPLAPCSRSTSESTAALGCLVKDYFPEPVTVSWNSGALTSGVHTFPAVLQSSGLYSLSSVVTVPSSSLGTKTYTCNVDHKPSNTKVDKRVESKYGPPCPPCPAPEFLGGPSVFLFPPKPKDTLMISRTPEVTCVVVDVSQEDPEVQFNWYVDGVEVHNAKTKPREEQFNSTYRVVSVLTVLHQDWLNGKEYKCKVSNKGLPSSIEKTISKAKGQPREPQVYTLPPSQEEMTKNQVSLTCLVKGFYPSDIAVEWESNGQPENNYKTTPPVLDSDGSFFLYSRLTVDKSRWQEGNVFSCSVMHEALHNHYTQKSLSLSLG

SEQ ID NO: 51 - protein, 215 aa, synthetic construct
  source 1..215: note = Synthetic
QSVLTQPPSASGTPGQRVTISCSGSSSNIGSNTVHWYQQLPGTAPKLLIYSDNQRPSGVPDRFSGSKSGTSASLAISGLQSEDEADYYCAAWDDSLNGVFGGGTKLTVLGQPKAAPSVTLFPPSSEELQANKATLVCLISDFYPGAVTVAWKADSSPVKAGVETTTPSKQSNNKYAASSYLSLTPEQWKSHRSYSCQVTHEGSTVEKTVAPTECS

SEQ ID NO: 52-70 - skipped (19 entries)

SEQ ID NO: 71 - protein, 17 aa, synthetic construct
  source 1..17: note = Synthetic
ESLIRFLEDPQQGGMDV

SEQ ID NO: 72 - protein, 10 aa, synthetic construct
  source 1..10: note = Synthetic
NSWTRSNNYI

SEQ ID NO: 73 - protein, 126 aa, synthetic construct
  source 1..126: note = Synthetic
QVQLQQSGAEVKKPGASVKVSCKASGYTFTSYYMHWVRQAPGQGLEWMGIINPSGGSTSYAQKFQGRVTMTRDTSTSTVYMELSSLRSEDTAVYYCARESLIRFLEDPQQGGMDVWGQGTTVTVSS

SEQ ID NO: 74 - protein, 121 aa, synthetic construct
  source 1..121: note = Synthetic
QSALTQPASVSGSPGQSLTISCTGTSSDIGGYNYVSWYQQHPGKAPKLIIYDVTDRPSGVSGRFSGSKSGNTASLTISGLQTEDEAEYFCNSWTRSNNYIFGGGTKLTVLGQPKAAPSVTL

SEQ ID NO: 75 - protein, 273 aa, synthetic construct
  source 1..273: note = Synthetic
QVQLQQSGAEVKKPGASVKVSCKASGYTFTSYYMHWVRQAPGQGLEWMGIINPSGGSTSYAQKFQGRVTMTRDTSTSTVYMELSSLRSEDTAVYYCARESLIRFLEDPQQGGMDVWGQGTTVTVSSGSASAPTLGGGGSGGGGSAAAQSALTQPASVSGSPGQSLTISCTGTSSDIGGYNYVSWYQQHPGKAPKLIIYDVTDRPSGVSGRFSGSKSGNTASLTISGLQTEDEAEYFCNSWTRSNNYIFGGGTKLTVLGQPKAAPSVTLFPPSS

SEQ ID NO: 76 - protein, 13 aa, synthetic construct
  source 1..13: note = Synthetic
DRYSSSWGGGFDY

SEQ ID NO: 77 - protein, 10 aa, synthetic construct
  source 1..10: note = Synthetic
QSYDASSLWV

SEQ ID NO: 78 - protein, 122 aa, synthetic construct
  source 1..122: note = Synthetic
EVQLVQSGGGVVQSGRSLRLSCVASGFSFSNYGMHWVRQAPGKGLEWLAFIWYDGSNKWYADSVKGRFTISRDNSKNALYLQMNSLRAEDTAVYYCARDRYSSSWGGGFDYWGQGTVLTVSS

SEQ ID NO: 79 - protein, 122 aa, synthetic construct
  source 1..122: note = Synthetic
NFMLTQPHSVSESPGRTVTIPCSGRGGSIASDSVQWYQQRPGSAPTTIIYEDNQRPSGVPDRFSGSVDSSSNSASLTISGLRTEDEADYYCQSYDASSLWVFGGKTKLTVLGQPKAAPSVTL

SEQ ID NO: 80 - protein, 275 aa, synthetic construct
  source 1..275: note = Synthetic
EVQLVQSGGGVVQSGRSLRLSCVASGFSFSNYGMHWVRQAPGKGLEWLAFIWYDGSNKWYADSVKGRFTISRDNSKNALYLQMNSLRAEDTAVYYCARDRYSSSWGGGFDYWGQGTVLTVSSGSASAPTLGGGGSGGGGSAAANFMLTQPHSVSESPGRTVTIPCSGRGGSIASDSVQWYQQRPGSAPTTIIYEDNQRPSGVPDRFSGSVDSSSNSASLTISGLRTEDEADYYCQSYDASSLWVFGGKTKLTVLGQPKAAPSVTLFPPSSKASGA

SEQ ID NO: 81 - protein, 10 aa, synthetic construct
  source 1..10: note = Synthetic
DRHSLGDFDY

SEQ ID NO: 82 - protein, 9 aa, synthetic construct
  source 1..9: note = Synthetic
QAWDSTTVV

SEQ ID NO: 83 - protein, 121 aa, synthetic construct
  source 1..121: note = Synthetic
QLQLQQSGGGLVKPGGSLRLSCAASGFTFSSYSMNWVRQAPGKGLEWVSSISSSSSYIYYADSVKGRFTISRDNAKNSLYLQMNSLRAEDTAVYYCVRDRHSLGDFDYWGQGTLVTVSSGS

SEQ ID NO: 84 - protein, 121 aa, synthetic construct
  source 1..121: note = Synthetic
SSELTQPSVSVSPGQTATITCSGDKLGDKYASWYQQKPGQSPVLVIYQDTKRPSGIPARFSGSNSGNTATLTISGTQAMDEAAYYCQAWDSTTVVFGGGTKLTVLGQPKAAPSVTLFPPSS

SEQ ID NO: 85 - protein, 201 aa, synthetic construct
  source 1..201: note = Synthetic
QLQLQQSGGGLVKPGGSLRLSCAASGFTFSSYSMNWVRQAPGKGLEWVSSISSSSSYIYYADSVKGRFTISRDNAKNSLYLQMNSLRAEDTAVYYCVRDRHSLGDFDYWGQGTLVTVSSGSASAPTLGGGGSGGGGSAAASSELTQPPSVSVSPGQTATITCSGDKLGDKYASWYQQKPGQSPVLVIYQDTKRPSGIPARF

SEQ ID NO: 86 - protein, 18 aa, synthetic construct
  source 1..18: note = Synthetic
HGLMDDSSGYYLSNAFDI

SEQ ID NO: 87 - protein, 11 aa, synthetic construct
  source 1..11: note = Synthetic
ATWDDSLTGVV

SEQ ID NO: 88 - protein, 129 aa, synthetic construct
  source 1..129: note = Synthetic
QVQLVQSGAEVKKPGSSVKVSCKASGGTFSSYAISWVRQAPGQGLEWMGGIIPIFGTANYAQKFQGRVTITADESTSTAYMELSSLRSEDTAVYYCANHGLMDDSSGYYLSNAFDIWGQGTMVTVSSGS

SEQ ID NO: 89 - protein, 126 aa, synthetic construct
  source 1..126: note = Synthetic
QPVLTQPPSASGTPGQRVTISCSGSSSNIGSNTVEWYQQLPGTAPKLLIHSNNQRPSGVPDRFSGSRSGTSASLAISGLQSEDEADYFCATWDDSLTGVVFGGGTTLTVLGQPKAAPSVTLFPPSS

SEQ ID NO: 90 - protein, 274 aa, synthetic construct
  source 1..274: note = Synthetic
QVQLVQSGAEVKKPGSSVKVSCKASGGTFSSYAISWVRQAPGQGLEWMGGIIPIFGTANYAQKFQGRVTITADESTSTAYMELSSLRSEDTAVYYCANHGLMDDSSGYYLSNAFDIWGQGTMVTVSSGSASAPTLGGGGSGGGGSAAAQPVLTQPPSASGTPGQRVTISCSGSSSNIGSNTVEWYQQLPGTAPKLLIHSNNQRPSGVPDRFSGSRSGTSASLAISGLQSEDEADYFCATWDDSLTGVVFGGGTTLTVLGQPKAAPSVTLFPPSS

SEQ ID NO: 91 - protein, 12 aa, synthetic construct
  source 1..12: note = Synthetic
VGTAAAGDAFDI

SEQ ID NO: 92 - protein, 11 aa, synthetic construct
  source 1..11: note = Synthetic
AAWDDSLSGWV

SEQ ID NO: 93 - protein, 123 aa, synthetic construct
  source 1..123: note = Synthetic
QVQLVQSGGGLIQPGGSLRLSCAASGFTVSSYSMNWVRQAPGKGLEWVSYISSSGSTIYYADSVKGRFTISRDNAKNSLYLQMNSLRAEDTALYYCAKVGTAAAGDAFDIWGQGTMVTVSSGS

SEQ ID NO: 94 - protein, 126 aa, synthetic construct
  source 1..126: note = Synthetic
QPVLTQPPSASGTPGQRVTISCFGSSSNIGSNYVYWYQQLPGTAPKLLIYRNNQRPSGVPDRFSGSKSGTSASLAISGLRSEDEADYYCAAWDDSLSGWVFGGGTKLTVLGQPKAAPSVTLFPPSS

SEQ ID NO: 95 - protein, 268 aa, synthetic construct
  source 1..268: note = Synthetic
QVQLVQSGGGLIQPGGSLRLSCAASGFTVSSYSMNWVRQAPGKGLEWVSYISSSGSTIYYADSVKGRFTISRDNAKNSLYLQMNSLRAEDTALYYCAKVGTAAAGDAFDIWGQGTMVTVSSGSASAPTLGGGGSGGGGSAAAQPVLTQPPSASGTPGQRVTISCFGSSSNIGSNYVYWYQQLPGTAPKLLIYRNNQRPSGVPDRFSGSKSGTSASLAISGLRSEDEADYYCAAWDDSLSGWVFGGGTKLTVLGQPKAAPSVTLFPPSS

SEQ ID NO: 96 - protein, 18 aa, synthetic construct
  source 1..18: note = Synthetic
VGFYDYVWGSYPYDAFDI

SEQ ID NO: 97 - protein, 9 aa, synthetic construct
  source 1..9: note = Synthetic
QQYGTSPLT

SEQ ID NO: 98 - protein, 127 aa, synthetic construct
  source 1..127: note = Synthetic
QIQLVQSGAEVKKPGASVKVSCKASGYTFTSYGISWVRQAPGQGLEWMGWISAYNGNTNYAQKLQGRVTMTTDTSTSTAYMELSSLRSEDTAVYYCARVGFYDYVWGSYPYDAFDIWGQGTMVTVSS

SEQ ID NO: 99 - protein, 108 aa, synthetic construct
  source 1..108: note = Synthetic
EIVMTQSPGTLSLSPGERATLSCRASQSVSSNYLAWYQQKPGQAPRLLIYDASNRATGIPARFSGSGSGTDFTLTISSLEPEDFALYYCQQYGTSPLTFGGGTKLEIK

SEQ ID NO: 100 - protein, 265 aa, synthetic construct
  source 1..265: note = Synthetic
QIQLVQSGAEVKKPGASVKVSCKASGYTFTSYGISWVRQAPGQGLEWMGWISAYNGNTNYAQKLQGRVTMTTDTSTSTAYMELSSLRSEDTAVYYCARVGFYDYVWGSYPYDAFDIWGQGTMVTVSSGSASAPTLGGGGSGGGGSAAAEIVMTQSPGTLSLSPGERATLSCRASQSVSSNYLAWYQQKPGQAPRLLIYDASNRATGIPARFSGSGSGTDFTLTISSLEPEDFALYYCQQYGTSPLTFGGGTKLEIKRTVAAPSVF

SEQ ID NO: 101 - protein, 14 aa, synthetic construct
  source 1..14: note = Synthetic
DTSNGGYSSSSFDY

SEQ ID NO: 102 - protein, 10 aa, synthetic construct
  source 1..10: note = Synthetic
SSYTSSSTLV

SEQ ID NO: 103 - protein, 123 aa, synthetic construct
  source 1..123: note = Synthetic
EVQLVQSGGGLVQPGRSLRLSCAASGFTFDDYAMHWVRQAPGKGLEWVSGISWNSGSIGYADSVKGRFTISRDNAKNSLYLQMNSLRAEDTALYYCAKDTSNGGYSSSSFDYWGQGTLVTVSS

SEQ ID NO: 104 - protein, 110 aa, synthetic construct
  source 1..110: note = Synthetic
QSALTQPASVSGSPGQSITISCTGTSSDVGGYNYVSWYQQHPGTAPKLMIYDVSYRPSGVSNRFSGSKSGNTASLTISGLQAEDEADYYCSSYTSSSTLVFGTGTKVTVL

SEQ ID NO: 105 - protein, 270 aa, synthetic construct
  source 1..270: note = Synthetic
EVQLVQSGGGLVQPGRSLRLSCAASGFTFDDYAMHWVRQAPGKGLEWVSGISWNSGSIGYADSVKGRFTISRDNAKNSLYLQMNSLRAEDTALYYCAKDTSNGGYSSSSFDYWGQGTLVTVSSGSASAPTLGGGGSGGGGSAAAQSALTQPASVSGSPGQSITISCTGTSSDVGGYNYVSWYQQHPGTAPKLMIYDVSYRPSGVSNRFSGSKSGNTASLTISGLQAEDEADYYCSSYTSSSTLVFGTGTKVTVLGQPKANPTVTLFPPSS

SEQ ID NO: 106 - protein, 15 aa, synthetic construct
  source 1..15: note = Synthetic
LVYGGYDEPGYYFDY

SEQ ID NO: 107 - protein, 11 aa, synthetic construct
  source 1..11: note = Synthetic
AAWDDSLNGWV

SEQ ID NO: 108 - protein, 124 aa, synthetic construct
  source 1..124: note = Synthetic
EVQLLESRAEVKKPGESLKISCKGSGYSFTSYWIGWVRQMPGKGPEWMGIIYPGDSDTRYSPSFQGQVTISADKSISTAYLQWSSLKASDTAMYYCARLVYGGYDEPGYYFDYWGQGTLVTVSS

SEQ ID NO: 109 - protein, 110 aa, synthetic construct
  source 1..110: note = Synthetic
QSVLTQPPSASGTPGQRVTISCSGSSSNIRSNTVNWYQQLPGTAPKLLIYSNNQRPSGVPDRFSGSKSGTSASLAISGLQSEDEADYYCAAWDDSLNGWVFGGGTKLTVL

SEQ ID NO: 110 - protein, 276 aa, synthetic construct
  source 1..276: note = Synthetic
EVQLLESRAEVKKPGESLKISCKGSGYSFTSYWIGWVRQMPGKGPEWMGIIYPGDSDTRYSPSFQGQVTISADKSISTAYLQWSSLKASDTAMYYCARLVYGGYDEPGYYFDYWGQGTLVTVSSGSASAPTLGGGGSGGGGSAAAQSVLTQPPSASGTPGQRVTISCSGSSSNIRSNTVNWYQQLPGTAPKLLIYSNNQRPSGVPDRFSGSKSGTSASLAISGLQSEDEADYYCAAWDDSLNGWVFGGGTKLTVLGQPKAAPSVTLFPPSSKASGA

SEQ ID NO: 111 - protein, 14 aa, synthetic construct
  source 1..14: note = Synthetic
VDGLEYSSGHNFDY

SEQ ID NO: 112 - protein, 10 aa, synthetic construct
  source 1..10: note = Synthetic
SSYAGSYTWV

SEQ ID NO: 113 - protein, 123 aa, synthetic construct
  source 1..123: note = Synthetic
EVQLVQSGGGLVQPGRSLRLSCAASGFTFDDYAMHWVRQAPGKGLEWVSGISWNSGSIGYADSVKGRFTISRDNSKNTLYLQMNSLRAEDTAVYYCAKVDGLEYSSGHNFDYWGQGTLVTVSS

SEQ ID NO: 114 - protein, 110 aa, synthetic construct
  source 1..110: note = Synthetic
QSALTQPPSVSGSPGQSVTISCTGSSSDVGYYDHVSWYQHHPGRAPKVIIYDVTKRPSGVPDRFSGSKSGNTASLTISGLQAEDEADYYCSSYAGSYTWVFGGGTELTVL

SEQ ID NO: 115 - protein, 270 aa, synthetic construct
  source 1..270: note = Synthetic
EVQLVQSGGGLVQPGRSLRLSCAASGFTFDDYAMHWVRQAPGKGLEWVSGISWNSGSIGYADSVKGRFTISRDNSKNTLYLQMNSLRAEDTAVYYCAKVDGLEYSSGHNFDYWGQGTLVTVSSGSASAPTLGGGGSGGGGSAAAQSALTQPPSVSGSPGQSVTISCTGSSSDVGYYDHVSWYQHHPGRAPKVIIYDVTKRPSGVPDRFSGSKSGNTASLTISGLQAEDEADYYCSSYAGSYTWVFGGGTELTVLGQPKAAPSVTLFPPSS

SEQ ID NO: 116 - protein, 179 aa, synthetic construct
  source 1..179: note = Synthetic
RELIDQYDVQRDDSSDGSLEDDDYHATTETIITMPTESDFLMQVDGKPKCCFFKFSSKIQYNKVVKAQLWIYLRPVETPTTVFVQILRLIKPMKDGTRYTGIRSLKLDMNPGTGIWQSIDVKTVLQNWLKQPESNLGIEIKALDENGHDLAVTFPGPGEDGLNPFLEVKVTDTPKRSRR